European Patent Application EP 4 241 790 A1, published September 13, 2023. Title: Expression System For The Treatment Of Cancer. Applicant: Fundacion para la Investigacion Medica Aplicada. The sequence listing filed with the application follows.

SEQUENCE LISTING (31 sequences)

SEQ ID NO: 1 - protein, 379 aa, Homo sapiens [sequence omitted]

SEQ ID NO: 2 - protein, 379 aa, Homo sapiens
  hSTING[H]wt
MPHSSLHPSIPCPRGHGAQKAALVLLSACLVTLWGLGEPPEHTLRYLVLHLASLQLGLLLNGVCSLAEELRHIHSRYRGSYWRTVRACLGCPLRRGALLLLSIYFYYSLPNAVGPPFTWMLALLGLSQALNILLGLKGLAPAEISAVCEKGNFNVAHGLAWSYYIGYLRLILPELQARIRTYNQHYNNLLRGAVSQRLYILLPLDCGVPDNLSMADPNIRFLDKLPQQTGDHAGIKDRVYSNSIYELLENGQRAGTCVLEYATPLQTLFAMSQYSQAGFSREDRLEQAKLFCRTLEDILADAPESQNNCRLIAYQEPADDSSFSLSQEVLRHLRQEEKEEVTVGSLKTSAVPSTSTMSQEPELLISGMEKPLPLRTDFS

SEQ ID NO: 3 - protein, 379 aa, Homo sapiens [sequence omitted]

SEQ ID NO: 4 - protein, 283 aa, Homo sapiens
  hSTING[H]truncated
MPHSSLHPSIPCPRGHGAQKAALVLLSACLVTLWGLGEPPEHTLRYLVLHLASLQLGLLLNGVCSLAEELRHIHSRYRGSYWRTVRACLGCPLRRGALLLLSIYFYYSLPNAVGPPFTWMLALLGLSQALNILLGLKGLAPAEISAVCEKGNFNVAHGLAWSYYIGYLRLILPELQARIRTYNQHYNNLLRGAVSQRLYILLPLDCGVPDNLSMADPNIRFLDKLPQQTGDHAGIKDRVYSNSIYELLENGQRNLQMTAASRCPRRFSGTCGRRKRKRLLWAA

SEQ ID NO: 5 - DNA, 1139 bp, Homo sapiens
  hSTING[R]-S162A/G230I/Q266I (hSTINGmut)
atgccccactccagcctgcatccatccatcccgtgtcccaggggtcacggggcccagaaggcagccttggttctgctgagtgcctgcctggtgaccctttgggggctaggagagccaccagagcacactctccggtacctggtgctccacctagcctccctgcagctgggactgctgttaaacggggtctgcagcctggctgaggagctgcgccacatccactccaggtaccggggcagctactggaggactgtgcgggcctgcctgggctgccccctccgccgtggggccctgttgctgctgtccatctatttctactactccctcccaaatgcggtcggcccgcccttcacttggatgcttgccctcctgggcctctcgcaggcactgaacatcctcctgggcctcaagggcctggccccagctgagatctctgcagtgtgtgaaaaagggaatttcaacgtggcccatgggctggcatgggcatattacatcggatatctgcggctgatcctgccagagctccaggcccggattcgaacttacaatcagcattacaacaacctgctacggggtgcagtgagccagcggctgtatattctcctcccattggactgtggggtgcctgataacctgagtatggctgaccccaacattcgcttcctggataaactgccccagcagaccattgaccgtgctggcatcaaggatcgggtttacagcaacagcatctatgagcttctggagaacgggcagcgggcgggcacctgtgtcctggagtacgccacccccttgatcactttgtttgccatgtcacaatacagtcaagctggctttagccgggaggataggcttgagcaggccaaactcttctgccggacacttgaggacatcctggcagatgcccctgagtctcagaacaactgccgcctcattgcctaccaggaacctgcagatgacagcagcttctcgctgtcccaggaggttctccggcacctgcggcaggaggaaaaggaagaggttactgtgggcagcttgaagacctcagcggtgcccagtacctccacgatgtcccaagagcctgagctcctcatcagtggaatggaaaagcccctccctctccgcacggatttctctta

SEQ ID NO: 6 - protein, 379 aa, Homo sapiens
  hSTING[R]-S162A/G230I/Q266I (hSTINGmut)
MPHSSLHPSIPCPRGHGAQKAALVLLSACLVTLWGLGEPPEHTLRYLVLHLASLQLGLLLNGVCSLAEELRHIHSRYRGSYWRTVRACLGCPLRRGALLLLSIYFYYSLPNAVGPPFTWMLALLGLSQALNILLGLKGLAPAEISAVCEKGNFNVAHGLAWAYYIGYLRLILPELQARIRTYNQHYNNLLRGAVSQRLYILLPLDCGVPDNLSMADPNIRFLDKLPQQTIDRAGIKDRVYSNSIYELLENGQRAGTCVLEYATPLITLFAMSQYSQAGFSREDRLEQAKLFCRTLEDILADAPESQNNCRLIAYQEPADDSSFSLSQEVLRHLRQEEKEEVTVGSLKTSAVPSTSTMSQEPELLISGMEKPLPLRTDFS

SEQ ID NO: 7 - DNA, 1137 bp, Mus musculus
  mSTINGwt
atgccatactccaacctgcatccagccatcccacggcccagaggtcaccgctccaaatatgtagccctcatctttctggtggccagcctgatgatcctttgggtggcaaaggatccaccaaatcacactctgaagtacctagcacttcacctagcctcgcacgaacttggactactgttgaaaaacctctgctgtctggctgaagagctgtgccatgtccagtccaggtaccagggcagctactggaaggctgtgcgcgcctgcctgggatgccccatccactgtatggctatgattctactatcgtcttatttctatttcctccaaaacactgctgacatatacctcagttggatgtttggccttctggtcctctataagtccctaagcatgctcctgggccttcagagcttgactccagcggaagtctctgcagtctgtgaagaaaagaagttaaatgttgcccacgggctggcctggtcatactacattgggtacttgcggttgatcttaccagggctccaggcccggatccgaatgttcaatcagctacataacaacatgctcagtggtgcagggagccgaagactgtacatcctctttccattggactgtggggtgcctgacaacctgagtgtagttgaccccaacattcgattccgagatatgctgccccagcaaaacatcgaccgtgctggcatcaagaatcgggtttattccaacagcgtctacgagattctggagaacggacagccagcaggcgtctgtatcctggagtacgccacccccttgcagaccctgtttgccatgtcacaggatgccaaagctggcttcagtcgggaggatcggcttgagcaggctaaactcttctgccggacacttgaggaaatcctggaagatgtccccgagtctcgaaataactgccgcctcattgtctaccaagaacccacagacggaaacagtttctcactgtctcaggaggtgctccggcacattcgtcaggaagaaaaggaggaggttaccatgaatgcccccatgacctcagtggcacctcctccctccgtactgtcccaagagccaagactcctcatcagtggtatggatcagcctctcccactccgcactgacctcatctga

SEQ ID NO: 8 - protein, 378 aa, Mus musculus
  mSTINGwt
MPYSNLHPAIPRPRGHRSKYVALIFLVASLMILWVAKDPPNHTLKYLALHLASHELGLLLKNLCCLAEELCHVQSRYQGSYWKAVRACLGCPIHCMAMILLSSYFYFLQNTADIYLSWMFGLLVLYKSLSMLLGLQSLTPAEVSAVCEEKKLNVAHGLAWSYYIGYLRLILPGLQARIRMFNQLHNNMLSGAGSRRLYILFPLDCGVPDNLSVVDPNIRFRDMLPQQNIDRAGIKNRVYSNSVYEILENGQPAGVCILEYATPLQTLFAMSQDAKAGFSREDRLEQAKLFCRTLEEILEDVPESRNNCRLIVYQEPTDGNSFSLSQEVLRHIRQEEKEEVTMNAPMTSVAPPPSVLSQEPRLLISGMDQPLPLRTDLI

SEQ ID NO: 9 - protein, 540 aa, Homo sapiens
  hIL-12sc
MCHQQLVISWFSLVFLASPLVAIWELKKDVYVVELDWYPDAPGEMVVLTCDTPEEDGITWTLDQSSEVLGSGKTLTIQVKEFGDAGQYTCHKGGEVLSHSLLLLHKKEDGIWSTDILKDQKEPKNKTFLRCEAKNYSGRFTCWWLTTISTDLTFSVKSSRGSSDPQGVTCGAATLSAERVRGDNKEYEYSVECQEDSACPAAEESLPIEVMVDAVHKLKYENYTSSFFIRDIIKPDPPKNLQLKPLKNSRQVEVSWEYPDTWSTPHSYFSLTFCVQVQGKSKREKKDRVFTDKTSATVICRKNASISVRAQDRYYSSSWSEWASVPCSGGGGSGGGGSGGGGSRNLPVATPDPGMFPCLHHSQNLLRAVSNMLQKARQTLEFYPCTSEEIDHEDITKDKTSTVEACLPLELTKNESCLNSRETSFITNGSCLASRKTSFMMALCLSSIYEDLKMYQVEFKTMNAKLLMDPKRQIFLDQNMLAVIDELMQALNFNSETVPQKSSLEEPDFYKTKIKLCILLHAFRIRAVTIDRVMSYLNAS

SEQ ID NO: 10 - protein, 543 aa, Mus musculus
  mIL-12sc
MGPQKLTISWFAIVLLVSPLMAMWELEKDVYVVEVDWTPDAPGETVNLTCDTPEEDDITWTSDQRHGVIGSGKTLTITVKEFLDAGQYTCHKGGETLSHSHLLLHKKENGIWSTEILKNFKNKTFLKCEAPNYSGRFTCSWLVQRNMDLKFNIKSSSSPPDSRAVTCGMASLSAEKVTLDQRDYEKYSVSCQEDVTCPTAEETLPIELALEARQQNKYENYSTSFFIRDIIKPDPPKNLQMKPLKNSQVEVSWEYPDSWSTPHSYFSLKFFVRIQRKKEKMKETEEGCNQKGAFLVEKTSTEVQCKGGNVCVQAQDRYYNSSCSKWACVPCRVRSGGGGSGGGGSGGGGSRVIPVSGPARCLSQSRNLLKTTDDMVKTAREKLKHYSCTAEDIDHEDITRDQTSTLKTCLPLELHKNESCLATRETSSTTRGSCLPPQKTSLMMTLCLGSIYEDLKMYQTEFQAINAALQNHNHQQIILDKGMLVAIDELMQSLNHNGETLRQKPPVGEADPYRVKMKLCILLHAFSTRVVTINRVMGYLSSA

SEQ ID NO: 11 - DNA, 13 bp, Homo sapiens
  ISRE
agtttcgctttct

SEQ ID NO: 12 - DNA, 212 bp, Homo sapiens
  ISREx4
atctctgcgatgaacctcacagtttcgctttctatctctgcgatgaacctcacagtttcgctttctatctctgcgatgaacctcacagtttcgctttctatctctgcgatgaacctcacagtttcgctttctgtgcctcttatgatctggatctcgagccatggtcgaggcctgtaggcgtgtacggtgggaggcttatataagcagagctc

SEQ ID NO: 13 - DNA, 156 bp, Homo sapiens
  ISREx4 short
gctagcagtttcgctttctgctagcagtttcgctttctgctagcagtttcgctttctgctagcagtttcgctttctgtgcctcttatgatctggatctcgagccatggtcgaggcctgtaggcgtgtacggtgggaggcttatataagcagagctc

SEQ ID NO: 14 - DNA, 22 bp, Homo sapiens
  miR122 target sequence
caaacaccattgtcacactcca

SEQ ID NO: 15 - DNA, 130 bp, Homo sapiens
  miR122 target sequence x5
atccaaacaccattgtcacactccaagaccaaacaccattgtcacactccaagaccaaacaccattgtcacactccaagaccaaacaccattgtcacactccaagaccaaacaccattgtcacactccac

SEQ ID NO: 16 - protein, 376 aa, Human herpesvirus 1
  thymidine kinase
MASYPGHQHASAFDQAARSRGHSNRRTALRPRRQQEATEVRPEQKMPTLLRVYIDGPHGMGKTTTTQLLVALGSRDDIVYVPEPMTYWRVLGASETIANIYTTQHRLDQGEISAGDAAVVMTSAQITMGMPYAVTDAVLAPHIGGEAGSSHAPPPALTIFLDRHPIAFMLCYPAARYLMGSMTPQAVLAFVALIPPTLPGTNIVLGALPEDRHIDRLAKRQRPGERLDLAMLAAIRRVYGLLANTVRYLQCGGSWREDWGQLSGTAVPPQGAEPQSNAGPRPHIGDTLFTLFRAPELLAPNGDLYNVFAWALDVLAKRLRSMHVFILDYDQSPAGCRDALLQLTSGMVQTHVTTPGSIPTICDLARTFAREMGEAN

SEQ ID NO: 17 - DNA, 103 bp, Adeno-associated virus - 8
  AAV ITR
catcatcaataatataccttattttggattgaagccaatatgataatgagggggtggagtttgtgacgtggcgcggggcgtgggaacggggcgggtgacgtag

SEQ ID NO: 18 - DNA, 219 bp, Mus musculus
  short IFNb A-promoter
caggagcttgaataaaatgaatattagaagctgttagaataagagaaaatgacagaggaaaactgaaagggagaactgaaagtgggaaattcctctgaggcagaaaggaccatcccttataaatagcacaggccatgaaggaagatcattctcactgcagcctttgacagcctttgcctcatcttgcaggtagcagccgacaccagcctggcttccatc

SEQ ID NO: 19 - DNA, 219 bp, Mus musculus
  short IFNb B-promoter
caggagcttgaataaaatgaatattagaagctgttagaataagagaaaatgacagaggaaaactgaaagggagaactgaaagcaaaaaattcctctgaggcagaaaggaccatcccttataaatagcacaggccatgaaggaagatcattctcactgcagcctttgacagcctttgcctcatcttgcaggtagcagccgacaccagcctggcttccatc

SEQ ID NO: 20 - DNA, 205 bp, Mus musculus
  short IFNb C-promoter
caggagcttgaataaaatgaatattagaagctgttagaataagagaaaatgacagaggaaaactgaaagggagaactgaaagtgggcagaaaggaccatcccttataaatagcacaggccatgaaggaagatcattctcactgcagcctttgacagcctttgcctcatcttgcaggtagcagccgacaccagcctggcttccatc

SEQ ID NO: 21 - DNA, 185 bp, Mus musculus
  short IFNb D-promoter
caggagcttgaataaaatgaatattagaagctgttagaataagagaaaatgacagaggaaaactgaaagggagaactgaaagtgggaaattcctctgaggcagaaaggaccatattctcactgcagcctttgacagcctttgcctcatcttgcaggtagcagccgacaccagcctggcttccatc

SEQ ID NO: 22 - DNA, 110 bp, Mus musculus
  short IFNb E-promoter
ggagaactgaaagtgggaaattcctctgaggcagaaagattctcactgcagcctttgacagcctttgcctcatcttgcaggtagcagccgacaccagcctggcttccatc

SEQ ID NO: 23 - DNA, 556 bp, Mus musculus
  CXCL9-promoter
gacacagacatctcgtgaaacatctggaaaaggtagcagggaacgggacagcagtagcttatgcaactaatctagcaattacaatgataggaaactgtagccacggtgagacgaaatggatttaccctcaacaaattaagaagctttgacttgtgaggaaaggcagtttgagtcgccatatagtgtcatgtcccacgtgggaagtacatctccaaccttcattgtacaacattaatatagtcattgtataatctattccacatccaggtagcaactttgcctgggggtggtttcacatcccttactataaactccccgtttatgtgaaatggaagtagaacatgcagaaattccctgggatctgagagtagggttttccccaggacgatcaatttgtggttagtttagttcttctaggtcagctgaggagaccagccaatcagagacgggaaggaaaagggatttcctaaataaatatgatccccaagaacatgctctctaaagacattctcggacttcactccaacacagtgactcaatagaactcagctctgcc

SEQ ID NO: 24 - DNA, 565 bp, Mus musculus
  CXCL10-promoter
tctaactgttcactaagttgtatagactttggatctggctaaatttggcgtgtgatttttttttaaagtttattccaagtattttataataaagcatatgaagtaaaaagcaaaaataaacagtgtaaacacaacaaatgtaaaaaccatggttagaacctgacttagatatcagttctgtgttttatttatgagagaaggaagatgagaattaaagccatttccagacttattctgcaaggcactgcatctgatttctcaaacagctcacgctttggaaagtgaaacttacctcactcgttaaaaattaaaaggagcacaagaggggagagggaaattccaagttcatgggtcacaataaacacaagcaatgccctcggtttacaggggacttccctcgggttgcggagccttgctgagtcatctccaaagtcagccaatcaggactcagggagggaaactctttgcagataaatactcctcagcagccggcactcgagaagcgcttcatccaccgctgagagacatcccgagccaaccttccggaagcctccccatcagcacc

SEQ ID NO: 25 - DNA, 571 bp, Mus musculus
  IFNb1-promoter
ccaggatgtggggttctctcccaaagggagctatggcccattgatgtgccatttctcttatagtacactattgtaagccccctgggagctcacagagaccctctcccaccatcccactatttcaaagggcagcagctgtgccatcctttcaggatgagcagctactctgcctggcttttcagtggacactttggctgtttgagagttcttttatcttcagggctgtctcctttctgttcttctctcctggatatttctcttcctttgctccagcaattggtgaaactgtacaagattttataaatccttagtttgtatatattttaacccagtacatagcatataaaatagccaggagcttgaataaaatgaatattagaagctgttagaataagagaaaatgacagaggaaaactgaaagggagaactgaaagtgggaaattcctctgaggcagaaaggaccatcccttataaatagcacaggccatgaaggaagatcattctcactgcagcctttgacagcctttgcctcatcttgcaggtagcagccgacaccagcctggcttccatc

SEQ ID NO: 26 - DNA, 202 bp, Mus musculus
  STATx4
atctctgcgatgaacctcacttcgctagaaatctctgcgatgaacctcacttcgctagaaatatctctgcgatgaacctcacttcgctagaaatctctgcgatgaacctcacttcgctagaagtgcctcttatgatctggatctcgagccatggtcgaggcctgtaggcgtgtacggtgggaggcttatataagcagagctc

SEQ ID NO: 27 - DNA, 208 bp, Mus musculus
  IRSF3x4
atctctgcgatgaacctcacgaaatagaaactatctctgcgatgaacctcacgaaatagaaactatctctgcgatgaacctcacgaaatagaaactatctctgcgatgaacctcacgaaatagaaactgtgcctcttatgatctggatctcgagccatggtcgaggcctgtaggcgtgtacggtgggaggcttatataagcagagctc

SEQ ID NO: 28 - DNA, 152 bp, Mus musculus
  short IRSF3x4
gctagcgaaatagaaactgctagcgaaatagaaactgctagcgaaatagaaactgctagcgaaatagaaactgtgcctcttatgatctggatctcgagccatggtcgaggcctgtaggcgtgtacggtgggaggcttatataagcagagctc

SEQ ID NO: 29 - DNA, 200 bp, Mus musculus
  NFκBx4
atctctgcgatgaacctcacgggactttccatctctgcgatgaacctcacgggactttccatctctgcgatgaacctcacgggactttccatctctgcgatgaacctcacgggactttccgtgcctcttatgatctggatctcgagccatggtcgaggcctgtaggcgtgtacggtgggaggcttatataagcagagctc

SEQ ID NO: 30 - DNA, 144 bp, Mus musculus
  short NFκBx4
gctagcgggactttccgctagcgggactttccgctagcgggactttccgctagcgggactttccgtgcctcttatgatctggatctcgagccatggtcgaggcctgtaggcgtgtacggtgggaggcttatataagcagagctc

SEQ ID NO: 31 - DNA, 581 bp, Mus musculus
  IFNb-minimal-promoter
ccccaggatgtggggttctctcccaaagggagctatggcccattgatgtgccatttctcttatagtacactattgtaagccccctgggagctcacagagaccctctcccaccatcccactatttcaaagggcagcagctgtgccatcctttcaggatgagcagctactctgcctggcttttcagtggacactttggctgtttgagagttcttttatcttcagggctgtctcctttctgttcttctctcctggatatttctcttcctttgctccagcaattggtgaaactgtacaagattttataaatccttagtttgtatatattttaacccagtacatagcatataaaatagcaggagcttgaataaaatgaatattagaagctgttagaataagagaaaatgacagaggaaaactgaaagggagaactgaaagtgggaaattcctctgaggcagaaaggaccatcccttataaatagcacaggccatgaaggaagatcattctcactgcagcctttgacagcctttgcctcatcttgcaggtagcagccgacaccagcctggcttccatcggatccatg